European Patent Specification EP 3 569 707 B1, published July 26, 2023. Title: High Rebaudioside C Content Stevia. Applicant: SUNTORY HOLDINGS LIMITED. The sequence listing filed with the application follows.

SEQUENCE LISTING (7 sequences)

SEQ ID NO: 1 - DNA, 60 bp, Stevia rebaudiana
gagtaaaatctataacgacactaaggtggaaaaagaatatgtaagccaattcgtagactt

SEQ ID NO: 2 - DNA, 60 bp, Stevia rebaudiana
gagtaaaatctataacgacactaaggtggaaaaagaatatgtaagccaattcgtagacta

SEQ ID NO: 3 - DNA, 25 bp, Artificial Sequence
  primer
tggtcaccctctaatcatgctaccg

SEQ ID NO: 4 - DNA, 46 bp, artificial
  primer
ttaactctcatgatcgatggcaaccgcacgcgcattcttttccaac

SEQ ID NO: 5 - DNA, 258 bp, Stevia rebaudiana
  misc_feature (258)..(258): The "n" at the position 258 may be "a" or "t".
tggtcaccctctaatcatgctaccgctttttggggaccaacctctgaatgctcgattactggaggacaaacaggtgggaatcgagataccaagaaatgaggaagatggttgcttgaccaaggagtcggttgctagatcactgaggtccgttgttgtggaaaacgaaggggagatctacaaggcgaacgcgagggagctgagtaaaatctataacgacactaaggtggaaaaagaatatgtaagccaattcgtagactn

SEQ ID NO: 6 - DNA, 258 bp, Stevia rebaudiana
tggtcaccctctaatcatgctaccgctttttggggaccaacctctgaatgctcgattactggaggacaaacaggtgggaatcgagataccaagaaatgaggaagatggttgcttgaccaaggagtcggttgctagatcactgaggtccgttgttgtggaaaacgaaggggagatctacaaggcgaacgcgagggagctgagtaaaatctataacgacactaaggtggaaaaagaatatgtaagccaattcgtagactt

SEQ ID NO: 7 - DNA, 258 bp, Stevia rebaudiana
tggtcaccctctaatcatgctaccgctttttggggaccaacctctgaatgctcgattactggaggacaaacaggtgggaatcgagataccaagaaatgaggaagatggttgcttgaccaaggagtcggttgctagatcactgaggtccgttgttgtggaaaacgaaggggagatctacaaggcgaacgcgagggagctgagtaaaatctataacgacactaaggtggaaaaagaatatgtaagccaattcgtagacta